European Patent Specification EP 4 323 545 B1, published October 29, 2025. Title: Optimized oligonucleotide TX probe for a multiplexing analysis of nucleic acids and a multiplexing method. Applicant: Biotype GmbH. The sequence listing filed with the application follows.

SEQUENCE LISTING (55 sequences)

SEQ ID NO: 1 - DNA, 22 bp, Artificial Sequence
  Primer for target Seq ID No. 12
  primer_bind (1)..(22)
ttggtggagtgatttgtctgct

SEQ ID NO: 2 - DNA, 21 bp, Artificial Sequence
  Primer for target Seq ID No. 12
  primer_bind (1)..(21)
tctaagggcatcacagacctg

SEQ ID NO: 3 - DNA, 25 bp, Artificial Sequence
  TX probe sequence
tcggcccttaaatagcccggtccgc

SEQ ID NO: 4 - DNA, 23 bp, Artificial Sequence
  TX probe sequence
actggacccagccgagcctttcc

SEQ ID NO: 5 - DNA, 25 bp, Artificial Sequence
  TX probe sequence
ccaaggtgatgtactcgctggccct

SEQ ID NO: 6 - DNA, 20 bp, Artificial Sequence
  TX probe sequence
gctggaattaccgcggctgc

SEQ ID NO: 7 - DNA, 25 bp, Artificial Sequence
  Primer for target Seq ID No. 10 and No. 11
tgttggggcatagttaaaacctgtg

SEQ ID NO: 8 - DNA, 21 bp, Artificial Sequence
  Primer for target Seq ID No. 10 and No. 11
tgtgttggcggatacccttcc

SEQ ID NO: 9 - DNA, 22 bp, Artificial Sequence
  TX probe sequence
cctgctgctcatccacaagacc

SEQ ID NO: 10 - DNA, 176 bp, Homo sapiens
  Target  sequence (1)..(176): NG_032903.2, REGION: 37880.. 38035
tgtgttggcggatacccttccataaaggctttaacacagaatcaaaagattcgataccataaggagttgctgcttcagccaaggcagcaatggccaaagcactgatggtccgaactttctgctgctcatccacaagacctacaaaaccaaacacaggttttaactatgccccaaca

SEQ ID NO: 11 - DNA, 176 bp, Homo sapiens
  Modified Target  sequence (1)..(176): NG_032903.2 REGION: 37880.. 38035 with substitution with Genomic Mutation ID COSV59208501
tgtgttggcggatacccttccataaaggctttaacacagaatcaaaagattcgataccataaggagttgctgcttcagccaaggcaggaatggccaaagcactgatggtccgaactttctgctgctcatccacaagacctacaaaaccaaacacaggttttaactatgccccaaca

SEQ ID NO: 12 - DNA, 155 bp, Aspergillus fumigatus Af293
  Target sequence (1)..(155): NC_007197 REGION: 443002..443156
ctaagggcatcacagacctgttattgccgcgcacttccatcggcttgagccgatagtccccctaagaagccagcggcccgcaaatgcggaccgggctatttaagggccgaggtctcgttcgttatcgcaattaagcagacaaatcactccaccaa

SEQ ID NO: 13 - DNA, 31 bp, Artificial Sequence
  Primer
  ENF1003 (1)..(31): EAC Code: ENF1003 no modification
  gene (1)..(31): ABL
  variation (1)..(31): no
tggagataacactctaagcataactaaaggt

SEQ ID NO: 14 - DNA, 28 bp, Artificial Sequence
  TX Probe
  ENPr1043 (1)..(28): EAC Code: ENPr1043 Modification No. 24 of table 2
  gene (1)..(28): ABL
  variation (1)..(28): no
ccatttttggtttgggcttcacaccatt

SEQ ID NO: 15 - DNA, 21 bp, Artificial Sequence
  Primer
  ENR1063 (1)..(21): EAC Code: ENR1063 no modification
  gene (1)..(21): ABL
  variation (1)..(21): no
gatgtagttgcttgggaccca

SEQ ID NO: 16 - DNA, 22 bp, Artificial Sequence
  Primer
  ENF701 (1)..(22): EAC Code: ENF701 no modification
  gene (1)..(22): AML1-ETO
  variation (1)..(22): t(8;21)(q22;q22)
cacctaccacagagccatcaaa

SEQ ID NO: 17 - DNA, 29 bp, Artificial Sequence
  TX Probe
  ENP747 (1)..(29): Modification No. 6 of table 2
  gene (1)..(29): AML1-ETO
  variation (1)..(29): t(8;21)(q22;q22)
aacctcgaaatcgtactgagaagcactcc

SEQ ID NO: 18 - DNA, 22 bp, Artificial Sequence
  Primer
  ENR761 (1)..(22): EAC Code: ENR761 no modification
  gene (1)..(22): AML1-ETO
  variation (1)..(22): t(8;21)(q22;q22)
atccacaggtgagtctggcatt

SEQ ID NO: 19 - DNA, 18 bp, Artificial Sequence
  Primer
  ENF402 (1)..(18): EAC Code: ENF402 no modification
  gene (1)..(18): BCR-ABL m-bcr
  variation (1)..(18): t(9;22)(q34;q11)
ctggcccaacgatggcga

SEQ ID NO: 20 - DNA, 21 bp, Artificial Sequence
  Primer
  ENF501 (1)..(21): EAC Code: ENF501 no modification
  gene (1)..(21): BCR-ABL M-bcr
  variation (1)..(21): t(9;22)(q34;q11)
tccgctgaccatcaayaagga

SEQ ID NO: 21 - DNA, 25 bp, Artificial Sequence
  TX Probe
  ENP541 (1)..(25): EAC Code: ENP541 Modification No. 17 of table 2
  gene (1)..(25): BCR-ABL M-bcr
  variation (1)..(25): t(9;22)(q34;q11)
cccttcagcggccagtagcatctga

SEQ ID NO: 22 - DNA, 21 bp, Artificial Sequence
  Primer
  ENR561 (1)..(21): EAC Code:ENR561 no modification
  gene (1)..(21): BCR-ABL M-bcr
  variation (1)..(21): t(9;22)(q34;q11)
cactcagaccctgaggctcaa

SEQ ID NO: 23 - DNA, 22 bp, Artificial Sequence
  Primer
  ENF803 (1)..(22): EAC Code:ENF803 no modification
  gene (1)..(22): CBFB-MYH11
  variation (1)..(22): inv(16)(p13q22)
cattagcacaacaggcctttga

SEQ ID NO: 24 - DNA, 22 bp, homo sapiens
  ENPr843 (1)..(22): EAC Code:ENPr843 Modification No. 21 of table 2
  gene (1)..(22): CBFB-MYH11A
  variation (1)..(22): inv(16)(p13q22)
tcgcgtgtccttctccgagcct

SEQ ID NO: 25 - DNA, 17 bp, Artificial Sequence
  Primer
  ENR862 (1)..(17): no modification
  gene (1)..(17): CBFB-MYH11 A
  variation (1)..(17): inv(16)(p13q22)
agggcccgcttggactt

SEQ ID NO: 26 - DNA, 19 bp, Artificial Sequence
  Primer
  ENF101 (1)..(19): no modification
  gene (1)..(19): E2A-PBX1
  variation (1)..(19): t(1;19)(q23;p13)
ccagcctcatgcacaacca

SEQ ID NO: 27 - DNA, 22 bp, Artificial Sequence
  TX Probe
  ENP141 (1)..(22): EAC Code: ENP141 Modification No. 18 of table 2
  gene (1)..(22): E2A-PBX1
  variation (1)..(22): t(1;19)(q23;p13)
ccctccctgacctgtctcggcc

SEQ ID NO: 28 - DNA, 21 bp, Artificial Sequence
  Primer
  ENR161 (1)..(21): EAC Code: ENR161 no modification
  gene (1)..(21): E2A-PBX1
  variation (1)..(21): t(1;19)(q23;p13)
gggctcctcggatactcaaaa

SEQ ID NO: 29 - DNA, 25 bp, Artificial Sequence
  Primer
  ENF207 (1)..(25): EAC Code: ENF207 no modification
  gene (1)..(25): MLL-AF4
  variation (1)..(25): t(4;11)(q21;q23)
cccaagtatccctgtaaaacaaaaa

SEQ ID NO: 30 - DNA, 23 bp, Artificial Sequence
  Primer
  ENF208 (1)..(23): EAC Code: ENF208 no modification
  gene (1)..(23): MLL-AF4
  variation (1)..(23): t(4;11)(q21;q23)
gatggagtccacaggatcagagt

SEQ ID NO: 31 - DNA, 22 bp, Artificial Sequence
  TX Probe
  ENP242 (1)..(22): EAC Code: ENP242 Modification No. 9 of tabel 2
  gene (1)..(22): MLL-AF4
  variation (1)..(22): t(4;11)(q21;q23)
catggccgcctcctttgacagc

SEQ ID NO: 32 - DNA, 22 bp, Artificial Sequence
  Primer
  ENR262 (1)..(22): EAC Code: ENR262 no modification
  gene (1)..(22): MLL-AF4
  variation (1)..(22): t(4;11)(q21;q23)
gaaaggaaacttggatggctca

SEQ ID NO: 33 - DNA, 19 bp, Artificial Sequence
  Primer
  ENF903 (1)..(19): EAC Code: ENF903 no modification
  gene (1)..(19): PML-RARA bcr1
  variation (1)..(19): t(15;17)(q22;q21)
tcttcctgcccaacagcaa

SEQ ID NO: 34 - DNA, 20 bp, Artificial Sequence
  TX Probe
  ENP942 (1)..(20): EAC Code: ENP942 Modification No. 8 of table 2
  gene (1)..(20): PML-RARA bcr1
  variation (1)..(20): t(15;17)(q22;q21)
agtgcccagccctccctcgc

SEQ ID NO: 35 - DNA, 21 bp, Artificial Sequence
  Primer
  ENR962 (1)..(21): EAC Code: ENR962 no modification
  gene (1)..(21): PML-RARA bcr1
  variation (1)..(21): t(15;17)(q22;q21)
gcttgtagatgcggggtagag

SEQ ID NO: 36 - DNA, 19 bp, Artificial Sequence
  Primer
  ENF301 (1)..(19): EAC Code: ENF301 no modification
  gene (1)..(19): TEL-AML1
  variation (1)..(19): t(12;21)(p13;q22)
ctctgtctccccgcctgaa

SEQ ID NO: 37 - DNA, 20 bp, Artificial Sequence
  TX Probe
  ENPr341 (1)..(20): EAC Code: ENPr341 Modification No. 7 of table 2
  gene (1)..(20): TEL-AML1
  variation (1)..(20): t(12;21)(p13;q22)
tcccaatgggcatggcgtgc

SEQ ID NO: 38 - DNA, 16 bp, Artificial Sequence
  Primer
  ENR361 (1)..(16): EAC Code: ENR361 no modification
  gene (1)..(16): TEL-AML1
  variation (1)..(16): t(12;21)(p13;q22)
cggctcgtgctggcat

SEQ ID NO: 39 - DNA, 19 bp, Artificial Sequence
  Primer
  ENF601 (1)..(19): EAC Code: ENF601 no modification
  gene (1)..(19): SIL-TAL1
  variation (1)..(19): del(1)(p32p32)
cgctcctaccctgcaaaca

SEQ ID NO: 40 - DNA, 22 bp, Artificial Sequence
  TX Probe
  ENP641 (1)..(22): EAC Code: ENP641 Modification No. 5 of table 2
  gene (1)..(22): SIL-TAL1
  variation (1)..(22): del(1)(p32p32)
acctcagctccgcggaagttgc

SEQ ID NO: 41 - DNA, 19 bp, Artificial Sequence
  Primer
  ENR664 (1)..(19): EAC Code: ENR664 no modification
  gene (1)..(19): SIL-TAL1
  variation (1)..(19): del(1)(p32p32)
ccgaggaagaggatgcaca

SEQ ID NO: 42 - DNA, 21 bp, Artificial Sequence
  Primer
  primer_bind (1)..(21)
gcaggcgcgcaaattacccaa

SEQ ID NO: 43 - DNA, 21 bp, Artificial Sequence
  Primer
  primer_bind (1)..(20)
cgcgcacttccatcggcttga

SEQ ID NO: 44 - DNA, 25 bp, Artificial Sequence
  TX probe Sequence
  variation (1)..(25): Modification No. 30 of table 4
acagattgagagctctttcttgatc

SEQ ID NO: 45 - DNA, 23 bp, Artificial Sequence
  TX Probe
  variation (1)..(23): Modification No. 29 of table 4
cgtagttgaaccttgggtctggc

SEQ ID NO: 46 - DNA, 27 bp, Artificial Sequenece
  TX Probe
  variation (1)..(27): Modification No. 37 of table 4
agattgtactcattccaattacgagac

SEQ ID NO: 47 - DNA, 21 bp, Artificial Sequence
  TX Probe
  variation (1)..(21): Modification No. 36 of table 4
aggtctcgttcgttatcgcaa

SEQ ID NO: 48 - DNA, 23 bp, Artificial Sequence
  TX Probe
  variation (1)..(23): Modification No. 28 of table 4
attgtcactacctccccgtgtcg

SEQ ID NO: 49 - DNA, 20 bp, Artificial Sequence
  TX Probe
  variation (1)..(20): Modification No. 31 of table 4
ccagccggaccagtactcgc

SEQ ID NO: 50 - DNA, 24 bp, Artificial Sequence
  TX Probe
  variation (1)..(24): Modification No. 38 of table 4
tgccctccaattgttcctcgttaa

SEQ ID NO: 51 - DNA, 23 bp, Artificial Sequence
  TX Probe
  variation (1)..(23): Modification No. 32 of table 4
caacaaaatagaaccgcacgtcc

SEQ ID NO: 52 - DNA, 22 bp, Artificial Sequence
  TX Probe
  variation (1)..(22): Modification No. 35 of table 4
tggtggagtgatttgtctgctt

SEQ ID NO: 53 - DNA, 22 bp, Artificial Sequence
  TX Probe
  variation (1)..(22): Modification No. 33 of table 4
tcttcgatcccctaactttcgt

SEQ ID NO: 54 - DNA, 22 bp, Artificial Sequence
  TX Probe
  variation (1)..(22): Modification No. 34 of table 4
ccttgtggtgcccttccgtcaa

SEQ ID NO: 55 - DNA, 992 bp, Aspergillus fumigatus
  gene (1)..(992): A. fumigatus Af293 NC_007197 REGION: 443029..4444020
  ref <301>: William C Niermann et al
  ref <302>: Genomic sequence of the pathogenic and allergenic filamentous fungus Aspergillus fumigatus
  ref <303>: Nature
  ref <304>: 438
  ref <305>: 22
  ref <306>: 1151-1156
  ref <307>: 2005-12-29
gcaggcgcgcaaattacccaatcccgacacggggaggtagtgacaataaatactgatacggggctcttttgggtctcgtaattggaatgagtacaatctaaatcccttaacgaggaacaattggagggcaagtctggtgccagcagccgcggtaattccagctccaatagcgtatattaaagttgttgcagttaaaaagctcgtagttgaaccttgggtctggctggccggtccgcctcaccgcgagtactggtccggctggacctttccttctggggaacctcatggccttcactggctgtggggggaaccaggacttttactgtgaaaaaattagagtgttcaaagcaggcctttgctcgaatacattagcatggaataatagaataggacgtgcggttctattttgttggtttctaggaccgccgtaatgattaatagggatagtcgggggcgtcagtattcagctgtcagaggtgaaattcttggatttgctgaagactaactactgcgaaagcattcgccaaggatgttttcattaatcagggaacgaaagttaggggatcgaagacgatcagataccgtcgtagtcttaaccataaactatgccgactagggatcgggcggtgtttctatgatgacccgctcggcaccttacgagaaatcaaagtttttgggttctggggggagtatggtcgcaaggctgaaacttaaagaaattgacggaagggcaccacaaggcgtggagcctgcggcttaatttgactcaacacggggaaactcaccaggtccagacaaaataaggattgacagattgagagctctttcttgatcttttggatggtggtgcatggccgttcttagttggtggagtgatttgtctgcttaattgcgataacgaacgagacctcggcccttaaatagcccggtccgcatttgcgggccgctggcttcttagggggactatcggctcaagccgatggaagtgcgcg